European Patent Specification EP 4 043 566 B1, published April 10, 2024. Title: Deoxyribozymes generating chemiluminescent signals. Applicant: Ustav organicke chemie a biochemie AV CR, v. v. i. The sequence listing filed with the application follows.

SEQUENCE LISTING (240 sequences)

SEQ ID NO: 1 - DNA, 32 bp, artificial
  general sequence of deoxyribozyme
  variation (1)..(1): G or T
  misc_feature (1)..(3): n is a, c, g, t or u
  variation (2)..(2): G or T
  variation (3)..(3): A or C
  variation (5)..(5): G or T
  misc_feature (5)..(18): n is a, c, g, t or u
  variation (6)..(6): A or T
  unsure (7)..(7)
  variation (8)..(8): G or T or A
  variation (9)..(9): A or C or G or T
  variation (10)..(10): A or G or T
  variation (11)..(11): T or C or A or G
  variation (12)..(12): A or T or G
  variation (13)..(13): A or T or G or C
  unsure (14)..(14): helix
  unsure (15)..(15)
  unsure (16)..(16): helix
  variation (17)..(17): T or A or C or G
  variation (18)..(18): G or A
  variation (23)..(23): T or C or G
  misc_feature (23)..(23): n is a, c, g, t or u
  variation (29)..(29): T or G or C
  misc_feature (29)..(32): n is a, c, g, t or u
  unsure (30)..(30): helix
  variation (31)..(31): G or A or C or T
  unsure (32)..(32)
nnnannnnnnnnnnnnnntgacntgggannnn

SEQ ID NO: 2 - DNA, 32 bp, artificial
  general sequence of deoxyribozyme
  variation (3)..(3): A or C
  misc_feature (3)..(3): n is a, c, g, t or u
  variation (6)..(6): A or T
  misc_feature (6)..(7): n is a, c, g, t or u
  unsure (7)..(7)
  variation (11)..(11): T or C
  misc_feature (11)..(11): n is a, c, g, t or u
  variation (13)..(13): A or T or G or C
  misc_feature (13)..(17): n is a, c, g, t or u
  unsure (14)..(14): helix
  unsure (15)..(15)
  unsure (16)..(16): helix
  variation (17)..(17): T or A or C or G
  variation (23)..(23): T or C
  misc_feature (23)..(23): n is a, c, g, t or u
  unsure (30)..(30): helix
  misc_feature (30)..(32): n is a, c, g, t or u
  variation (31)..(31): G or A or C or T
  unsure (32)..(32)
ggnagnngaanannnnngtgacntgggatnnn

SEQ ID NO: 3 - DNA, 32 bp, artificial
  general sequence of deoxyribozyme
  unsure (7)..(7)
  misc_feature (7)..(7): n is a, c, g, t or u
  variation (13)..(13): A or T or G or C
  misc_feature (13)..(17): n is a, c, g, t or u
  unsure (14)..(14): helix
  unsure (15)..(15)
  unsure (16)..(16): helix
  variation (17)..(17): T or A or C or G
  unsure (30)..(30): helix
  misc_feature (30)..(30): n is a, c, g, t or u
  unsure (32)..(32)
  misc_feature (32)..(32): n is a, c, g, t or u
ggaagangaatannnnngtgacttgggatngn

SEQ ID NO: 4 - DNA, 31 bp, artificial
  pool sequence
  unsure (16)..(16): 70 nucleotides
  misc_feature (16)..(16): n is a, c, g, t or u
ggaagagatggcgacnagctgatcctgatgg

SEQ ID NO: 5 - DNA, 15 bp, artificial
  blocking oligonucleotide BO1, REV1
ccatcaggatcagct

SEQ ID NO: 6 - DNA, 23 bp, artificial
  short oligonucleotide, FWD1
gaattctaatacgactcactata

SEQ ID NO: 7 - DNA, 33 bp, artificial
  splint oligonucleotide
gtcgccatctcttcctatagtgagtcgtattag

SEQ ID NO: 8 - DNA, 100 bp, artificial
  deoxyribozyme
ggaagagatggcgacgacacagggacgatgccgaatatcctcagtgcgcagggccgcaggggggagtgacttgggatggggggtcagctgatcctgatgg

SEQ ID NO: 9 - DNA, 105 bp, artificial
  library sequence
ggaagagatggcgacgacacagggacgatgccgaatatcctcagtgcgcagggccgcaggggggagtgacttgggatggggggtccactaatgatctgcccgatg

SEQ ID NO: 10 - DNA, 20 bp, artificial
  blocking oligonucleotide BO2, REV2
catcgggcagatcattagtg

SEQ ID NO: 11 - DNA, 20 bp, artificial
  short oligonucleotide
accgctcaggtgtagtatca

SEQ ID NO: 12 - DNA, 35 bp, artificial
  splint oligonucleotide
gtcgccatctcttcctgatactacacctgagcggt

SEQ ID NO: 13 - DNA, 20 bp, artificial
  FWD2
accgctcaggtgtagtatca

SEQ ID NO: 14 - DNA, 40 bp, artificial
  deoxyribozyme consensus sequence
  unsure (7)..(7): 26 nucleotides
  misc_feature (7)..(7): n is a, c, g, t or u
  unsure (18)..(18): 18 nucleotides
  misc_feature (18)..(18): n is a, c, g, t or u
ggaagangaatatccccnggggagtgacttgggatggggg

SEQ ID NO: 15 - DNA, 105 bp, artificial
  deoxyribozyme
ggaagatatggcgcgaacaaatggacaatgccgaatatcccccgcacgcagggcaacaagggggagtgacttgggatgggggctgcactaatgatctgcccgatg

SEQ ID NO: 16 - DNA, 105 bp, artificial
  deoxyribozyme
ggaagaaatgacgaggccacacggacgaggctgaatatcctcactgcggtgtgccccagggaggagtgacttgggatggtgggttcactaatgatctgcccgatg

SEQ ID NO: 17 - DNA, 105 bp, artificial
  deoxyribozyme
ggaagatagtgtgtcgataaagggacaatgctgaatttcctccctgagccggcgcgtaggggggagtgacttgggatggggggtgcactaatgatctgcccgatg

SEQ ID NO: 18 - DNA, 105 bp, artificial
  deoxyribozyme
ggaagacttgacgagcgcacagcgcttgttcagaatatcacccgtcatgtgttcgtgaagggggagtgacttgggatgggggttccactaatgatctgcccgatg

SEQ ID NO: 19 - DNA, 104 bp, artificial
  deoxyribozyme
ggaagaaatggtgcgacacaggggcgctccagaatatcctcattgcgatatgccgcagggaggagtgacttgggatggtgggtccactaatgatctgcccgatg

SEQ ID NO: 20 - DNA, 105 bp, artificial
  deoxyribozyme
ggaagaaatgtagaggaaacagtgactctgcagaatatcctcactgcgtagtggggcaggggggagtgacttgggatgggggctacactaatgatctgcccgatg

SEQ ID NO: 21 - DNA, 104 bp, artificial
  deoxyribozyme
ggaagaaacgcgacgacacagtaatgatgcggaatatccccccttcatagggcgaaaggggggagtgacttgggatgggggttacactaatgatctgcccgatg

SEQ ID NO: 22 - DNA, 105 bp, artificial
  deoxyribozyme
ggcagagatggcaacgtcaacatgaggatgccgcatatccccagtgcacacttgggcagtggggagtgacttgggatgggggaaacactaatgatctgcccgatg

SEQ ID NO: 23 - DNA, 105 bp, artificial
  deoxyribozyme
ggaagatatggcggtgactcttcgaagctgccgaatatcccccgtgcgcggagcctcaggggggagtgacttgggatggggggtccactaatgatctgcccgatg

SEQ ID NO: 24 - DNA, 105 bp, artificial
  deoxyribozyme
ggaagaaatgccgacctcccagggtggaggctgaatatccaccatggtccggaacggatgggggagtgacttgggatgggggaaccactaatgatctgcccgatg

SEQ ID NO: 25 - DNA, 46 bp, artificial
  minimized catalytic core
ggaagaaaaagaatatccccaaaaggggagtgacttgggatggggg

SEQ ID NO: 26 - DNA, 46 bp, artificial
  deoxyribozyme
ggaagaaaaagaatatcctcaaaaggggagtgacttgggatggggg

SEQ ID NO: 27 - DNA, 46 bp, artificial
  deoxyribozyme
ggaagaaaaagaatatccccaaaagaggagtgacttgggatggggg

SEQ ID NO: 28 - DNA, 46 bp, artificial
  deoxyribozyme
ggaagaaaaagaatatccccaaaaggggagtgacttgggatggtgg

SEQ ID NO: 29 - DNA, 46 bp, artificial
  deoxyribozyme
ggaagaaaaagaatatcctcaaaagaggagtgacttgggatggggg

SEQ ID NO: 30 - DNA, 46 bp, artificial
  deoxyribozyme
ggaagaaaaagaatatcctcaaaaggggagtgacttgggatggtgg

SEQ ID NO: 31 - DNA, 46 bp, artificial
  deoxyribozyme
ggaagaaaaagaatatccccaaaagaggagtgacttgggatggtgg

SEQ ID NO: 32 - DNA, 46 bp, artificial
  deoxyribozyme
ggaagaaaaagaatatcctcaaaagaggagtgacttgggatggtgg

SEQ ID NO: 33 - DNA, 46 bp, artificial
  deoxyribozyme
tgaagaaaaagaatatccccaaaaggggagtgacttgggatggggg

SEQ ID NO: 34 - DNA, 46 bp, artificial
  deoxyribozyme
gtaagaaaaagaatatccccaaaaggggagtgacttgggatggggg

SEQ ID NO: 35 - DNA, 46 bp, artificial
  deoxyribozyme
ggcagaaaaagaatatccccaaaaggggagtgacttgggatggggg

SEQ ID NO: 36 - DNA, 46 bp, artificial
  deoxyribozyme
ggaataaaaagaatatccccaaaaggggagtgacttgggatggggg

SEQ ID NO: 37 - DNA, 46 bp, artificial
  deoxyribozyme
ggaagtaaaagaatatccccaaaaggggagtgacttgggatggggg

SEQ ID NO: 38 - DNA, 46 bp, artificial
  deoxyribozyme
ggaagaaaaataatatccccaaaaggggagtgacttgggatggggg

SEQ ID NO: 39 - DNA, 46 bp, artificial
  deoxyribozyme
ggaagaaaaaaaatatccccaaaaggggagtgacttgggatggggg

SEQ ID NO: 40 - DNA, 46 bp, artificial
  deoxyribozyme
ggaagaaaaagcatatccccaaaaggggagtgacttgggatggggg

SEQ ID NO: 41 - DNA, 46 bp, artificial
  deoxyribozyme
ggaagaaaaaggatatccccaaaaggggagtgacttgggatggggg

SEQ ID NO: 42 - DNA, 46 bp, artificial
  deoxyribozyme
ggaagaaaaagtatatccccaaaaggggagtgacttgggatggggg

SEQ ID NO: 43 - DNA, 46 bp, artificial
  deoxyribozyme
ggaagaaaaagattatccccaaaaggggagtgacttgggatggggg

SEQ ID NO: 44 - DNA, 46 bp, artificial
  deoxyribozyme
ggaagaaaaagagtatccccaaaaggggagtgacttgggatggggg

SEQ ID NO: 45 - DNA, 46 bp, artificial
  deoxyribozyme
ggaagaaaaagaaaatccccaaaaggggagtgacttgggatggggg

SEQ ID NO: 46 - DNA, 46 bp, artificial
  deoxyribozyme
ggaagaaaaagaacatccccaaaaggggagtgacttgggatggggg

SEQ ID NO: 47 - DNA, 46 bp, artificial
  deoxyribozyme
ggaagaaaaagaagatccccaaaaggggagtgacttgggatggggg

SEQ ID NO: 48 - DNA, 46 bp, artificial
  deoxyribozyme
ggaagaaaaagaatttccccaaaaggggagtgacttgggatggggg

SEQ ID NO: 49 - DNA, 46 bp, artificial
  deoxyribozyme
ggaagaaaaagaatgtccccaaaaggggagtgacttgggatggggg

SEQ ID NO: 50 - DNA, 46 bp, artificial
  deoxyribozyme
ggaagaaaaagaatatccccaaaaggggaatgacttgggatggggg

SEQ ID NO: 51 - DNA, 46 bp, artificial
  deoxyribozyme
ggaagaaaaagaatatccccaaaaggggagtgacctgggatggggg

SEQ ID NO: 52 - DNA, 46 bp, artificial
  deoxyribozyme
ggaagaaaaagaatatccccaaaaggggagtgacgtgggatggggg

SEQ ID NO: 53 - DNA, 46 bp, artificial
  deoxyribozyme
ggaagaaaaagaatatccccaaaaggggagtgacttgggagggggg

SEQ ID NO: 54 - DNA, 46 bp, artificial
  deoxyribozyme
ggaagaaaaagaatatccccaaaaggggagtgacttgggacggggg

SEQ ID NO: 55 - DNA, 46 bp, artificial
  deoxyribozyme
ggaagaaaaagaatatccccaaaaggggagtgacttgggatggggt

SEQ ID NO: 56 - DNA, 46 bp, artificial
  deoxyribozyme
ggaagaaaaagaatatccccaaaaggggagtgacttgggatgggga

SEQ ID NO: 57 - DNA, 46 bp, artificial
  deoxyribozyme
ggaagaaaaagaatatccccaaaaggggagtgacttgggatggggc

SEQ ID NO: 58 - DNA, 46 bp, artificial
  deoxyribozyme
ggaagaaaaagaataaccccaaaaggggtgtgacttgggatggggg

SEQ ID NO: 59 - DNA, 46 bp, artificial
  deoxyribozyme
ggaagaaaaagaatacccccaaaaggggggtgacttgggatggggg

SEQ ID NO: 60 - DNA, 46 bp, artificial
  deoxyribozyme
ggaagaaaaagaatagccccaaaaggggcgtgacttgggatggggg

SEQ ID NO: 61 - DNA, 46 bp, artificial
  deoxyribozyme
ggaagaaaaagaatattcccaaaagggaagtgacttgggatagggg

SEQ ID NO: 62 - DNA, 46 bp, artificial
  deoxyribozyme
ggaagaaaaagaatattcccaaaagggaagtgacttgggattgggg

SEQ ID NO: 63 - DNA, 46 bp, artificial
  deoxyribozyme
ggaagaaaaagaatatctccaaaaggagagtgacttgggatgaggg

SEQ ID NO: 64 - DNA, 46 bp, artificial
  deoxyribozyme
ggaagaaaaagaatatctccaaaaggagagtgacttgggatgtggg

SEQ ID NO: 65 - DNA, 46 bp, artificial
  deoxyribozyme
ggaagaaaaagaatatcctcaaaagaggagtgacttgggatggagg

SEQ ID NO: 66 - DNA, 46 bp, artificial; identical to SEQ ID NO: 32
  deoxyribozyme

SEQ ID NO: 67 - DNA, 46 bp, artificial
  deoxyribozyme
ggaagaaaaagaatatccctaaaaagggagtgacttgggatgggag

SEQ ID NO: 68 - DNA, 46 bp, artificial
  deoxyribozyme
ggaagaaaaagaatatccctaaaaagggagtgacttgggatgggtg

SEQ ID NO: 69 - DNA, 46 bp, artificial
  deoxyribozyme
ggaagaaaaagaatatctttaaaaaaagagtgacttgggatgaaag

SEQ ID NO: 70 - DNA, 46 bp, artificial
  deoxyribozyme
ggaagaaaaagaatatctttaaaaaaagagtgacttgggatgtttg

SEQ ID NO: 71 - DNA, 46 bp, artificial
  deoxyribozyme
ggaagaaaaagaatatttttaaaaaaaaagtgacttgggataaaag

SEQ ID NO: 72 - DNA, 46 bp, artificial
  deoxyribozyme
ggaagaaaaagaatatttttaaaaaaaaagtgacttgggatttttg

SEQ ID NO: 73 - DNA, 43 bp, artificial
  deoxyribozyme
ggaagaaaaagaatatcccaaaagggagtgacttgggatgggg

SEQ ID NO: 74 - DNA, 40 bp, artificial
  deoxyribozyme
ggaagaaaaagaatatccaaaaggagtgacttgggatggg

SEQ ID NO: 75 - DNA, 37 bp, artificial
  deoxyribozyme
ggaagaaaaagaatatcaaaagagtgacttgggatgg

SEQ ID NO: 76 - DNA, 46 bp, artificial
  deoxyribozyme
ggaagaaaaagaatatacccaaaaggggagtgacttgggatggggg

SEQ ID NO: 77 - DNA, 46 bp, artificial
  deoxyribozyme
ggaagaaaaagaatatgcccaaaaggggagtgacttgggatggggg

SEQ ID NO: 78 - DNA, 46 bp, artificial
  deoxyribozyme
ggaagaaaaagaatattcccaaaaggggagtgacttgggatggggg

SEQ ID NO: 79 - DNA, 46 bp, artificial
  deoxyribozyme
ggaagaaaaagaatatacccaaaagggaagtgacttgggatagggg

SEQ ID NO: 80 - DNA, 46 bp, artificial
  deoxyribozyme
ggaagaaaaagaatatccccaaaagggaagtgacttgggatagggg

SEQ ID NO: 81 - DNA, 46 bp, artificial
  deoxyribozyme
ggaagaaaaagaatatgcccaaaagggaagtgacttgggatagggg

SEQ ID NO: 82 - DNA, 46 bp, artificial
  deoxyribozyme
ggaagaaaaagaatatacccaaaagggaagtgacttgggattgggg

SEQ ID NO: 83 - DNA, 46 bp, artificial
  deoxyribozyme
ggaagaaaaagaatatccccaaaagggaagtgacttgggattgggg

SEQ ID NO: 84 - DNA, 46 bp, artificial
  deoxyribozyme
ggaagaaaaagaatatgcccaaaagggaagtgacttgggattgggg

SEQ ID NO: 85 - DNA, 46 bp, artificial
  deoxyribozyme
ggaagaaaaagaatatccccaaaaggggagtgacttgggatagggg

SEQ ID NO: 86 - DNA, 46 bp, artificial
  deoxyribozyme
ggaagaaaaagaatatccccaaaaggggagtgacttgggattgggg

SEQ ID NO: 87 - DNA, 46 bp, artificial
  deoxyribozyme
ggaagaaaaagaatattcccaaaagggaagtgacttgggatggggg

SEQ ID NO: 88 - DNA, 46 bp, artificial
  deoxyribozyme
ggaagaaaaagaatattcccaaaaggggagtgacttgggattgggg

SEQ ID NO: 89 - DNA, 46 bp, artificial
  deoxyribozyme
ggaagaaaaagaatatgcccaaaaggggagtgacttgggatcgggg

SEQ ID NO: 90 - DNA, 46 bp, artificial
  deoxyribozyme
ggaagaaaaagaatatccccaaaagggcagtgacttgggatggggg

SEQ ID NO: 91 - DNA, 46 bp, artificial
  deoxyribozyme
ggaagaaaaagaatatccccaaaagggaagtgacttgggatggggg

SEQ ID NO: 92 - DNA, 46 bp, artificial
  deoxyribozyme
ggaagaaaaagaatatcaccaaaaggggagtgacttgggatggggg

SEQ ID NO: 93 - DNA, 46 bp, artificial
  deoxyribozyme
ggaagaaaaagaatatcgccaaaaggggagtgacttgggatggggg

SEQ ID NO: 94 - DNA, 46 bp, artificial
  deoxyribozyme
ggaagaaaaagaatatctccaaaaggggagtgacttgggatggggg

SEQ ID NO: 95 - DNA, 46 bp, artificial
  deoxyribozyme
ggaagaaaaagaatatcaccaaaaggagagtgacttgggatgaggg

SEQ ID NO: 96 - DNA, 46 bp, artificial
  deoxyribozyme
ggaagaaaaagaatatccccaaaaggagagtgacttgggatgaggg

SEQ ID NO: 97 - DNA, 46 bp, artificial
  deoxyribozyme
ggaagaaaaagaatatcgccaaaaggagagtgacttgggatgaggg

SEQ ID NO: 98 - DNA, 46 bp, artificial
  deoxyribozyme
ggaagaaaaagaatatcaccaaaaggagagtgacttgggatgtggg

SEQ ID NO: 99 - DNA, 46 bp, artificial
  deoxyribozyme
ggaagaaaaagaatatccccaaaaggagagtgacttgggatgtggg

SEQ ID NO: 100 - DNA, 46 bp, artificial
  deoxyribozyme
ggaagaaaaagaatatcgccaaaaggagagtgacttgggatgtggg

SEQ ID NO: 101 - DNA, 46 bp, artificial
  deoxyribozyme
ggaagaaaaagaatatccccaaaaggggagtgacttgggatgaggg

SEQ ID NO: 102 - DNA, 46 bp, artificial
  deoxyribozyme
ggaagaaaaagaatatccccaaaaggggagtgacttgggatgtggg

SEQ ID NO: 103 - DNA, 46 bp, artificial
  deoxyribozyme
ggaagaaaaagaatatctccaaaaggagagtgacttgggatggggg

SEQ ID NO: 104 - DNA, 46 bp, artificial
  deoxyribozyme
ggaagaaaaagaatatctccaaaaggggagtgacttgggatgtggg

SEQ ID NO: 105 - DNA, 46 bp, artificial
  deoxyribozyme
ggaagaaaaagaatatcgccaaaaggggagtgacttgggatgcggg

SEQ ID NO: 106 - DNA, 46 bp, artificial
  deoxyribozyme
ggaagaaaaagaatatccccaaaaggcgagtgacttgggatggggg

SEQ ID NO: 107 - DNA, 46 bp, artificial
  deoxyribozyme
ggaagaaaaagaatatccccaaaaggagagtgacttgggatggggg

SEQ ID NO: 108 - DNA, 46 bp, artificial
  deoxyribozyme
ggaagaaaaagaatatccacaaaaggggagtgacttgggatggggg

SEQ ID NO: 109 - DNA, 46 bp, artificial
  deoxyribozyme
ggaagaaaaagaatatccgcaaaaggggagtgacttgggatggggg

SEQ ID NO: 110 - DNA, 46 bp, artificial
  deoxyribozyme
ggaagaaaaagaatatccacaaaagaggagtgacttgggatggagg

SEQ ID NO: 111 - DNA, 46 bp, artificial
  deoxyribozyme
ggaagaaaaagaatatccccaaaagaggagtgacttgggatggagg

SEQ ID NO: 112 - DNA, 46 bp, artificial
  deoxyribozyme
ggaagaaaaagaatatccgcaaaagaggagtgacttgggatggagg

SEQ ID NO: 113 - DNA, 46 bp, artificial
  deoxyribozyme
ggaagaaaaagaatatccacaaaagaggagtgacttgggatggtgg

SEQ ID NO: 114 - DNA, 46 bp, artificial
  deoxyribozyme
ggaagaaaaagaatatccgcaaaagaggagtgacttgggatggtgg

SEQ ID NO: 115 - DNA, 46 bp, artificial
  deoxyribozyme
ggaagaaaaagaatatccccaaaaggggagtgacttgggatggagg

SEQ ID NO: 116 - DNA, 46 bp, artificial
  deoxyribozyme
ggaagaaaaagaatatccgcaaaaggggagtgacttgggatggcgg

SEQ ID NO: 117 - DNA, 46 bp, artificial
  deoxyribozyme
ggaagaaaaagaatatccccaaaagcggagtgacttgggatggggg

SEQ ID NO: 118 - DNA, 46 bp, artificial
  deoxyribozyme
ggaagaaaaagaatatcccaaaaaggggagtgacttgggatggggg

SEQ ID NO: 119 - DNA, 46 bp, artificial
  deoxyribozyme
ggaagaaaaagaatatcccgaaaaggggagtgacttgggatggggg

SEQ ID NO: 120 - DNA, 46 bp, artificial
  deoxyribozyme
ggaagaaaaagaatatccctaaaaggggagtgacttgggatggggg

SEQ ID NO: 121 - DNA, 46 bp, artificial
  deoxyribozyme
ggaagaaaaagaatatcccaaaaaagggagtgacttgggatgggag

SEQ ID NO: 122 - DNA, 46 bp, artificial
  deoxyribozyme
ggaagaaaaagaatatccccaaaaagggagtgacttgggatgggag

SEQ ID NO: 123 - DNA, 46 bp, artificial
  deoxyribozyme
ggaagaaaaagaatatcccgaaaaagggagtgacttgggatgggag

SEQ ID NO: 124 - DNA, 46 bp, artificial
  deoxyribozyme
ggaagaaaaagaatatcccaaaaaagggagtgacttgggatgggtg

SEQ ID NO: 125 - DNA, 46 bp, artificial
  deoxyribozyme
ggaagaaaaagaatatccccaaaaagggagtgacttgggatgggtg

SEQ ID NO: 126 - DNA, 46 bp, artificial
  deoxyribozyme
ggaagaaaaagaatatcccgaaaaagggagtgacttgggatgggtg

SEQ ID NO: 127 - DNA, 46 bp, artificial
  deoxyribozyme
ggaagaaaaagaatatccccaaaaggggagtgacttgggatgggag

SEQ ID NO: 128 - DNA, 46 bp, artificial
  deoxyribozyme
ggaagaaaaagaatatccccaaaaggggagtgacttgggatgggtg

SEQ ID NO: 129 - DNA, 46 bp, artificial
  deoxyribozyme
ggaagaaaaagaatatccctaaaaagggagtgacttgggatggggg

SEQ ID NO: 130 - DNA, 46 bp, artificial
  deoxyribozyme
ggaagaaaaagaatatcccaaaaatgggagtgacttgggatgggag

SEQ ID NO: 131 - DNA, 46 bp, artificial
  deoxyribozyme
ggaagaaaaagaatatcccgaaaacgggagtgacttgggatgggag

SEQ ID NO: 132 - DNA, 46 bp, artificial
  deoxyribozyme
ggaagaaaaagaatatccctaaaaggggagtgacttgggatgggtg

SEQ ID NO: 133 - DNA, 46 bp, artificial
  deoxyribozyme
ggaagaaaaagaatatcccgaaaatgggagtgacttgggatgggag

SEQ ID NO: 134 - DNA, 46 bp, artificial
  deoxyribozyme
ggaagaaaaagaatatcccgaaaaggggagtgacttgggatgggcg

SEQ ID NO: 135 - DNA, 46 bp, artificial
  deoxyribozyme
ggaagaaaaagaatatccccaaaacgggagtgacttgggatggggg

SEQ ID NO: 136 - DNA, 46 bp, artificial
  deoxyribozyme
ggaagaaaaagaatatccccaaaaagggagtgacttgggatggggg

SEQ ID NO: 137 - DNA, 46 bp, artificial
  deoxyribozyme
ggaagaaaaagaatttcctcaaaaggggagtgacttgggatggggg

SEQ ID NO: 138 - DNA, 46 bp, artificial
  deoxyribozyme
ggcagaaaaagcatatccccaaaaggggagtgacttgggatggggg

SEQ ID NO: 139 - DNA, 46 bp, artificial
  deoxyribozyme
ggaagaaaaagcatatcctcaaaaggggagtgacttgggatggggg

SEQ ID NO: 140 - DNA, 46 bp, artificial
  deoxyribozyme
ggaagaaaaagaatatccgcaaaaggggagtgacttgggatggcga

SEQ ID NO: 141 - DNA, 46 bp, artificial
  deoxyribozyme
ggaagaaaaagatagtaaccaaaaggggagtgacttgggatggggg

SEQ ID NO: 142 - DNA, 46 bp, artificial
  deoxyribozyme
ggaagaaaaagcatatccccaaaaggggagtgacttgggatggggt

SEQ ID NO: 143 - DNA, 46 bp, artificial
  deoxyribozyme
ggaagaaaaagaatatcctcaaaaggggagtgacttgggatggggt

SEQ ID NO: 144 - DNA, 46 bp, artificial
  deoxyribozyme
ggaagtaaaagaatatcctcaaaaggggagtgacttgggatggggt

SEQ ID NO: 145 - DNA, 46 bp, artificial
  deoxyribozyme
ggaagaaaaagtatatcctcaaaaggggagtgacttgggatggggg

SEQ ID NO: 146 - DNA, 46 bp, artificial
  deoxyribozyme
ggaagaaaaagcatatccacaaaaggggagtgacttgggatggggg

SEQ ID NO: 147 - DNA, 46 bp, artificial
  deoxyribozyme
ggcagtaaaagcatatccacaaaaggggagtgacttgggatggggg

SEQ ID NO: 148 - DNA, 46 bp, artificial
  deoxyribozyme
ggaagaaaaaggatatcctcaaaaggggagtgacttgggatggggg

SEQ ID NO: 149 - DNA, 46 bp, artificial
  deoxyribozyme
ggaagtaaaagcatatcctcaaaaggggagtgacttgggatggggg

SEQ ID NO: 150 - DNA, 46 bp, artificial
  deoxyribozyme
ggaagaaaaagaatatcatcaaaaggggagtgacttgggatggggg

SEQ ID NO: 151 - DNA, 46 bp, artificial
  deoxyribozyme
ggaagaaaaatatctaccctaaaaggggagtgacttgggatggggg

SEQ ID NO: 152 - DNA, 46 bp, artificial
  deoxyribozyme
ggaagaaaaagcatatccccaaaaggggagtgacttgggatgaggg

SEQ ID NO: 153 - DNA, 46 bp, artificial
  deoxyribozyme
ggaagaaaaagaatatcctcaaaaggggagtgacttgggatagggg

SEQ ID NO: 154 - DNA, 46 bp, artificial
  deoxyribozyme
ggaagaaaaaggatatccacaaaaggggagtgacttgggatggggg

SEQ ID NO: 155 - DNA, 46 bp, artificial
  deoxyribozyme
ggaagaaaaagcatatcctcaaaagaggagtgacttgggatggtgg

SEQ ID NO: 156 - DNA, 46 bp, artificial
  deoxyribozyme
ggcagaaaaagaatatcctcaaaaggggagtgacttgggatggggg

SEQ ID NO: 157 - DNA, 46 bp, artificial
  deoxyribozyme
ggaagtaaaagaatatcaccaaaaggggagtgacttgggatggggg

SEQ ID NO: 158 - DNA, 46 bp, artificial
  deoxyribozyme
ggaagaaaaagaacatcctcaaaaggggagtgacttgggatggggg

SEQ ID NO: 159 - DNA, 46 bp, artificial
  deoxyribozyme
ggaagaaaaagcatatacccaaaaggggagtgacttgggatggggg

SEQ ID NO: 160 - DNA, 46 bp, artificial
  deoxyribozyme
ggaagaaaaagcgtatacccaaaaggggagtgacttgggatggggc

SEQ ID NO: 161 - DNA, 46 bp, artificial
  deoxyribozyme
ggaagtaaaagaatttccccaaaaggggagtgacttgggatggggg

SEQ ID NO: 162 - DNA, 46 bp, artificial
  deoxyribozyme
ggaagaaaaagaatatcctcaaaaggggagtgacttgggatgggga

SEQ ID NO: 163 - DNA, 46 bp, artificial
  deoxyribozyme
ggaagaaaaagaatatccttaaaagaggagtgacttgggatggtgg

SEQ ID NO: 164 - DNA, 46 bp, artificial
  deoxyribozyme
ggcagaaaaagaatatccccaaaaggggaatgacttgggatggggg

SEQ ID NO: 165 - DNA, 46 bp, artificial
  deoxyribozyme
ggaagaaaaagaatattctcaaaaggggagtgacttgggatgaggg

SEQ ID NO: 166 - DNA, 46 bp, artificial
  deoxyribozyme
ggaagaaaaagaatttccccaaaagggaagtgacttgggattgggg

SEQ ID NO: 167 - DNA, 43 bp, artificial
  deoxyribozyme
  unsure (7)..(7): 3 nucleotides
  misc_feature (7)..(7): n is a, c, g, or t
ggaagangaatatccccaaaaggggagtgacttgggatggggg

SEQ ID NO: 168 - DNA, 43 bp, artificial; identical to SEQ ID NO: 167
  deoxyribozyme
  unsure (7)..(7): 10 nucleotides
  misc_feature (7)..(7): n is a, c, g, or t

SEQ ID NO: 169 - DNA, 43 bp, artificial; identical to SEQ ID NO: 167
  deoxyribozyme
  unsure (7)..(7): 30 nucleotides
  misc_feature (7)..(7): n is a, c, g, or t

SEQ ID NO: 170 - DNA, 43 bp, artificial
  deoxyribozyme
  unsure (21)..(21): 3 nucleotides
  misc_feature (21)..(21): n is a, c, g, or t
ggaagaaaaagaatatccccnggggagtgacttgggatggggg

SEQ ID NO: 171 - DNA, 43 bp, artificial; identical to SEQ ID NO: 170
  deoxyribyzme
  unsure (21)..(21): 10 nucleotides
  misc_feature (21)..(21): n is a, c, g, or t

SEQ ID NO: 172 - DNA, 43 bp, artificial; identical to SEQ ID NO: 170
  deoxyribozyme
  unsure (21)..(21): 30 nucleotides
  misc_feature (21)..(21): n is a, c, g, or t

SEQ ID NO: 173 - DNA, 47 bp, artificial
  deoxyribozyme
  unsure (47)..(47): 3 nucleotides
  misc_feature (47)..(47): n is a, c, g, or t
ggaagaaaaagaatatccccaaaaggggagtgacttgggatgggggn

SEQ ID NO: 174 - DNA, 47 bp, artificial; identical to SEQ ID NO: 173
  deoxyribozyme
  unsure (47)..(47): 10 nucleotides
  misc_feature (47)..(47): n is a, c, g, or t

SEQ ID NO: 175 - DNA, 47 bp, artificial; identical to SEQ ID NO: 173
  deoxyribozyme
  unsure (47)..(47): 30 nucleotides
  misc_feature (47)..(47): n is a, c, g, or t

SEQ ID NO: 176 - DNA, 45 bp, artificial
  deoxyribozyme
ggaagaagagaatatccccaaaaggggagtgacttgggatggggg

SEQ ID NO: 177 - DNA, 45 bp, artificial
  deoxyribozyme
ggaagaactgaatatccccaaaaggggagtgacttgggatggggg

SEQ ID NO: 178 - DNA, 45 bp, artificial
  deoxyribozyme
ggaagataagaatatccccaaaaggggagtgacttgggatggggg

SEQ ID NO: 179 - DNA, 45 bp, artificial
  deoxyribozyme
ggaagaaccgaatatccccaaaaggggagtgacttgggatggggg

SEQ ID NO: 180 - DNA, 45 bp, artificial
  deoxyribozyme
ggaagaccagaatatccccaaaaggggagtgacttgggatggggg

SEQ ID NO: 181 - DNA, 52 bp, artificial
  deoxyribozyme
ggaagagggatgaccagaatatccccaaaaggggagtgacttgggatggggg

SEQ ID NO: 182 - DNA, 52 bp, artificial
  deoxyribozyme
ggaagaacgtaatcgggaatatccccaaaaggggagtgacttgggatggggg

SEQ ID NO: 183 - DNA, 52 bp, artificial
  deoxyribozyme
ggaagacctcgctaccgaatatccccaaaaggggagtgacttgggatggggg

SEQ ID NO: 184 - DNA, 52 bp, artificial
  deoxyribozyme
ggaagagggggatcttgaatatccccaaaaggggagtgacttgggatggggg

SEQ ID NO: 185 - DNA, 52 bp, artificial
  deoxyribozyme
ggaagattaacgtctcgaatatccccaaaaggggagtgacttgggatggggg

SEQ ID NO: 186 - DNA, 72 bp, artificial
  deoxyribozyme
ggaagacgcccgctgttttacagtgctgcaaaaaacgaatatccccaaaaggggagtgacttgggatggggg

SEQ ID NO: 187 - DNA, 72 bp, artificial
  deoxyribozyme
ggaagaagtctggccgtcgaatctggcctatgtattgaatatccccaaaaggggagtgacttgggatggggg

SEQ ID NO: 188 - DNA, 72 bp, artificial
  deoxyribozyme
ggaagacataagagtggtggcgaccgttacaattaggaatatccccaaaaggggagtgacttgggatggggg

SEQ ID NO: 189 - DNA, 72 bp, artificial
  deoxyribozyme
ggaagaaatgggctcgaattaacgggtagttaattagaatatccccaaaaggggagtgacttgggatggggg

SEQ ID NO: 190 - DNA, 72 bp, artificial
  deoxyribozyme
ggaagaaggtgataggggagcgcacggaattacccagaatatccccaaaaggggagtgacttgggatggggg

SEQ ID NO: 191 - DNA, 45 bp, artificial
  deoxyribozyme
ggaagaaaaagaatatccccggaggggagtgacttgggatggggg

SEQ ID NO: 192 - DNA, 45 bp, artificial
  deoxyribozyme
ggaagaaaaagaatatccccgagggggagtgacttgggatggggg

SEQ ID NO: 193 - DNA, 45 bp, artificial
  deoxyribozyme
ggaagaaaaagaatatcccctaaggggagtgacttgggatggggg

SEQ ID NO: 194 - DNA, 45 bp, artificial
  deoxyribozyme
ggaagaaaaagaatatccccgctggggagtgacttgggatggggg

SEQ ID NO: 195 - DNA, 45 bp, artificial
  deoxyribozyme
ggaagaaaaagaatatccccaatggggagtgacttgggatggggg

SEQ ID NO: 196 - DNA, 52 bp, artificial
  deoxyribozyme
ggaagaaaaagaatatccccgggaaggcctggggagtgacttgggatggggg

SEQ ID NO: 197 - DNA, 52 bp, artificial
  deoxyribozyme
ggaagaaaaagaatatccccttttactgtgggggagtgacttgggatggggg

SEQ ID NO: 198 - DNA, 52 bp, artificial
  deoxyribozyme
ggaagaaaaagaatatcccccttagcaaatggggagtgacttgggatggggg

SEQ ID NO: 199 - DNA, 52 bp, artificial
  deoxyribozyme
ggaagaaaaagaatatccccaaaaagcatgggggagtgacttgggatggggg

SEQ ID NO: 200 - DNA, 52 bp, artificial
  deoxyribozyme
ggaagaaaaagaatatccccaatttcacccggggagtgacttgggatggggg

SEQ ID NO: 201 - DNA, 72 bp, artificial
  deoxyribozyme
ggaagaaaaagaatatcccctaacgagtctcaaaagctacttcgctataaggggagtgacttgggatggggg

SEQ ID NO: 202 - DNA, 72 bp, artificial
  deoxyribozyme
ggaagaaaaagaatatccccgggtgacaccaccgataacgagccttaaacggggagtgacttgggatggggg

SEQ ID NO: 203 - DNA, 72 bp, artificial
  deoxyribozyme
ggaagaaaaagaatatcccccgaccaccaacccaagtagacattatgagtggggagtgacttgggatggggg

SEQ ID NO: 204 - DNA, 72 bp, artificial
  deoxyribozyme
ggaagaaaaagaatatcccctggctccctccaagggtaggcattcacgagggggagtgacttgggatggggg

SEQ ID NO: 205 - DNA, 72 bp, artificial
  deoxyribozyme
ggaagaaaaagaatatccccgcagtgtagtgagaggacctcagcacacgcggggagtgacttgggatggggg

SEQ ID NO: 206 - DNA, 49 bp, artificial
  deoxyribozyme
ggaagaaaaagaatatccccaaaaggggagtgacttgggatggggggat

SEQ ID NO: 207 - DNA, 49 bp, artificial
  deoxyribozyme
ggaagaaaaagaatatccccaaaaggggagtgacttgggatgggggtgg

SEQ ID NO: 208 - DNA, 49 bp, artificial
  deoxyribozyme
ggaagaaaaagaatatccccaaaaggggagtgacttgggatgggggtgt

SEQ ID NO: 209 - DNA, 49 bp, artificial
  deoxyribozyme
ggaagaaaaagaatatccccaaaaggggagtgacttgggatggggggcg

SEQ ID NO: 210 - DNA, 49 bp, artificial; identical to SEQ ID NO: 207
  deoxyribozyme

SEQ ID NO: 211 - DNA, 56 bp, artificial
  deoxyribozyme
ggaagaaaaagaatatccccaaaaggggagtgacttgggatgggggacctaggcaa

SEQ ID NO: 212 - DNA, 56 bp, artificial
  deoxyribozyme
ggaagaaaaagaatatccccaaaaggggagtgacttgggatgggggtgttcatcaa

SEQ ID NO: 213 - DNA, 56 bp, artificial
  deoxyribozyme
ggaagaaaaagaatatccccaaaaggggagtgacttgggatggggggatagactct

SEQ ID NO: 214 - DNA, 56 bp, artificial
  deoxyribozyme
ggaagaaaaagaatatccccaaaaggggagtgacttgggatgggggatacccttgt

SEQ ID NO: 215 - DNA, 56 bp, artificial
  deoxyribozyme
ggaagaaaaagaatatccccaaaaggggagtgacttgggatgggggcgatctgacg

SEQ ID NO: 216 - DNA, 76 bp, artificial
  deoxyribozyme
ggaagaaaaagaatatccccaaaaggggagtgacttgggatgggggcgaagttggcaaacattataagttggggag

SEQ ID NO: 217 - DNA, 76 bp, artificial
  deoxyribozyme
ggaagaaaaagaatatccccaaaaggggagtgacttgggatgggggcaaggactttatacaatgctcgcgggtcga

SEQ ID NO: 218 - DNA, 76 bp, artificial
  deoxyribozyme
ggaagaaaaagaatatccccaaaaggggagtgacttgggatgggggtggagcatgcattcttggacaaaatcttgt

SEQ ID NO: 219 - DNA, 76 bp, artificial
  deoxyribozyme
ggaagaaaaagaatatccccaaaaggggagtgacttgggatggggggtgctacttaaattctgtgtgtgactttaa

SEQ ID NO: 220 - DNA, 76 bp, artificial
  deoxyribozyme
ggaagaaaaagaatatccccaaaaggggagtgacttgggatgggggttggctgccgtcccaggcggcacgatagac

SEQ ID NO: 221 - DNA, 50 bp, artificial
  deoxyribozyme
ggaagatcctgaatatccccttgaggggagtgacttgggatgggggctag

SEQ ID NO: 222 - DNA, 50 bp, artificial
  deoxyribozyme
ggaagagaacgaatatccccacctggggagtgacttgggatgggggcgaa

SEQ ID NO: 223 - DNA, 50 bp, artificial
  deoxyribozyme
ggaagatgccgaatatccccgtcgggggagtgacttgggatgggggtacg

SEQ ID NO: 224 - DNA, 50 bp, artificial
  deoxyribozyme
ggaagagcgagaatatccccacagggggagtgacttgggatgggggacgg

SEQ ID NO: 225 - DNA, 50 bp, artificial
  deoxyribozyme
ggaagaccctgaatatccccccgtggggagtgacttgggatggggggctc

SEQ ID NO: 226 - DNA, 68 bp, artificial
  deoxyribozyme
ggaagactttacctacgaatatccccgtaggcactcggggagtgacttgggatgggggacgctcccat

SEQ ID NO: 227 - DNA, 68 bp, artificial
  deoxyribozyme
ggaagatcgatgaggcgaatatccccagatcacctaggggagtgacttgggatgggggagcggcaccg

SEQ ID NO: 228 - DNA, 68 bp, artificial
  deoxyribozyme
ggaagactccttttatgaatatccccctgtctttaaggggagtgacttgggatgggggcagatcgcta

SEQ ID NO: 229 - DNA, 68 bp, artificial
  deoxyribozyme
ggaagatcgaccgccagaatatcccctcagcgcgagggggagtgacttgggatgggggagaaggaagt

SEQ ID NO: 230 - DNA, 68 bp, artificial
  deoxyribozyme
ggaagataacgtaggggaatatccccccagaaggtaggggagtgacttgggatgggggccccggacgt

SEQ ID NO: 231 - DNA, 68 bp, artificial
  deoxyribozyme
ggaagaaaaagaatatcccccaatcgtgcggggagtgacttgggatgggggaagcacgattgaccttc

SEQ ID NO: 232 - DNA, 15 bp, artificial
  target
gaaggtcaatcgtgc

SEQ ID NO: 233 - DNA, 68 bp, artificial
  deoxyribozyme
ggaagaaaaagaatatccccctcttaagaggggagtgacttgggatgggggaatcttaagagaaggga

SEQ ID NO: 234 - DNA, 15 bp, artificial
  target
tcccttctcttaaga

SEQ ID NO: 235 - DNA, 68 bp, artificial
  deoxyribozyme
ggaagaaaaagaatatccccggcactgatggggagtgacttgggatgggggaaatcagtgcccagtgg

SEQ ID NO: 236 - DNA, 15 bp, artificial
  target
ccactgggcactgat

SEQ ID NO: 237 - DNA, 68 bp, artificial
  deoxyribozyme
ggaagaaaaagaatatccccatgatcggaggggagtgacttgggatgggggaatccgatcatccgaag

SEQ ID NO: 238 - DNA, 15 bp, artificial
  target
cttcggatgatcgga

SEQ ID NO: 239 - DNA, 68 bp, artificial
  deoxyribozyme
ggaagaaaaagaatatccccagtaatagcggggagtgacttgggatgggggaagctattacttatctt

SEQ ID NO: 240 - DNA, 15 bp, artificial
  target
aagataagtaatagc